European Patent Application EP 4 748 927 A2, published May 27, 2026. Title: MODIFIED TRANSPOSASES FOR IMPROVED INSERTION SEQUENCE BIAS. Applicant: Illumina, Inc. Application EP, filed January 26, 2025. The sequence listing filed with the application follows.

SEQUENCE LISTING (26 sequences)

SEQ ID NO: 1 - protein, 476 aa, unidentified
  REGION 1..476: note = Transposase Tn5
MITSALHRAADWAKSVFSSAALGDPRRTARLVNVAAQLAKYSGKSITISSEGSEAMQEGAYRFIRNPNVSAEAIRKAGAMQTVKLAQEFPELLAIEDTTSLSYRHQVAEELGKLGSIQDKSRGWWVHSVLLLEATTFRTVGLLHQEWWMRPDDPADADEKESGKWLAAAATSRLRMGSMMSNVIAVCDREADIHAYLQDKLAHNERFVVRSKHPRKDVESGLYLYDHLKNQPELGGYQISIPQKGVVDKRGKRKNRPARKASLSLRSGRITLKQGNITLNAVLAEEINPPKGETPLKWLLLTSEPVESLAQALRVIDIYTHRWRIEEFHKAWKTGAGAERQRMEEPDNLERMVSILSFVAVRLLQLRESFTLPQALRAQGLLKEAEHVESQSAETVLTPDECQLLGYLDKGKRKRKEKAGSLQWAYMAIARLGGFMDSKRTGIASWGALWEGWEALQSKLDGFLAAKDLMAQGIKI

SEQ ID NO: 2 - protein, 476 aa, unidentified
  REGION 1..476: note = Transposase Tn5
  SITE 248: note = Variant - X = Y, T, K, S, L, A, W, P, G, R, F, H
MITSALHRAADWAKSVFSSAALGDPRRTARLVNVAAQLAKYSGKSITISSEGSEAMQEGAYRFIRNPNVSAEAIRKAGAMQTVKLAQEFPELLAIEDTTSLSYRHQVAEELGKLGSIQDKSRGWWVHSVLLLEATTFRTVGLLHQEWWMRPDDPADADEKESGKWLAAAATSRLRMGSMMSNVIAVCDREADIHAYLQDKLAHNERFVVRSKHPRKDVESGLYLYDHLKNQPELGGYQISIPQKGVVXKRGKRKNRPARKASLSLRSGRITLKQGNITLNAVLAEEINPPKGETPLKWLLLTSEPVESLAQALRVIDIYTHRWRIEEFHKAWKTGAGAERQRMEEPDNLERMVSILSFVAVRLLQLRESFTLPQALRAQGLLKEAEHVESQSAETVLTPDECQLLGYLDKGKRKRKEKAGSLQWAYMAIARLGGFMDSKRTGIASWGALWEGWEALQSKLDGFLAAKDLMAQGIKI

SEQ ID NO: 3 - protein, 476 aa, unidentified
  REGION 1..476: note = Transposase Tn5
  SITE 119: note = Variant - X = L, M, S, A, V
MITSALHRAADWAKSVFSSAALGDPRRTARLVNVAAQLAKYSGKSITISSEGSEAMQEGAYRFIRNPNVSAEAIRKAGAMQTVKLAQEFPELLAIEDTTSLSYRHQVAEELGKLGSIQXKSRGWWVHSVLLLEATTFRTVGLLHQEWWMRPDDPADADEKESGKWLAAAATSRLRMGSMMSNVIAVCDREADIHAYLQDKLAHNERFVVRSKHPRKDVESGLYLYDHLKNQPELGGYQISIPQKGVVDKRGKRKNRPARKASLSLRSGRITLKQGNITLNAVLAEEINPPKGETPLKWLLLTSEPVESLAQALRVIDIYTHRWRIEEFHKAWKTGAGAERQRMEEPDNLERMVSILSFVAVRLLQLRESFTLPQALRAQGLLKEAEHVESQSAETVLTPDECQLLGYLDKGKRKRKEKAGSLQWAYMAIARLGGFMDSKRTGIASWGALWEGWEALQSKLDGFLAAKDLMAQGIKI

SEQ ID NO: 4 - protein, 476 aa, unidentified
  REGION 1..476: note = Transposase Tn5
MITSALHRAADWAKSVFSSAALGDPRRTARLVNVAAQLAKYSGKSITISSEGSEAMQEGAYRFIRNPNVSAEAIRKAGAMQTVKLAQEFPELLAIEDTTSLSYRHQVAEELGKLGSIQDKSRGWMVHSVLLLEATTFRTVGLLHQEWWMRPDDPADADEKESGKWLAAAATSRLRMGSMMSNVIAVCDREADIHAYLQDKLAHNERFVVRSKHPRKDVESGLYLYDHLKNQPELGGYQISIPQKGVVDKRGKRKNRPARKASLSLRSGRITLKQGNITLNAVLAEEINPPKGETPLKWLLLTSEPVESLAQALRVIDIYTHRWRIEEFHKAWKTGAGAERQRMEEPDNLERMVSILSFVAVRLLQLRESFTLPQALRAQGLLKEAEHVESQSAETVLTPDECQLLGYLDKGKRKRKEKAGSLQWAYMAIARLGGFMDSKRTGIASWGALWEGWEALQSKLDGFLAAKDLMAQGIKI

SEQ ID NO: 5 - protein, 477 aa, unidentified
  REGION 1..477: note = Transposase Tn5
MITSALHRAADWAKSVFSSAALGDPRRTARLVNVAAQLAKYSGKSITISSEGSEAMQEGAYRFIRNPNVSAEAIRKAGAMQTVKLAQEFPELLAIEDTTSLSYRHQVAEELGKLGSIQDKSRGWWVHSVLLLEATTFRTVGLLHQEWWMRPDDPADADEKESGKWLAAAATSRLRMGSMMSNVIAVCDREADIHAYLQDKLAHNERFVVRSKHPRKDVESGLYLYDHLKNQPELGGYQISIPQKGVVDVKRGKRKNRPARKASLSLRSGRITLKQGNITLNAVLAEEINPPKGETPLKWLLLTSEPVESLAQALRVIDIYTHRWRIEEFHKAWKTGAGAERQRMEEPDNLERMVSILSFVAVRLLQLRESFTLPQALRAQGLLKEAEHVESQSAETVLTPDECQLLGYLDKGKRKRKEKAGSLQWAYMAIARLGGFMDSKRTGIASWGALWEGWEALQSKLDGFLAAKDLMAQGIKI

SEQ ID NO: 6 - protein, 476 aa, unidentified
  REGION 1..476: note = Transposase Tn5
  SITE 120: note = Variant - X = Y, F, W, E
MITSALHRAADWAKSVFSSAALGDPRRTARLVNVAAQLAKYSGKSITISSEGSEAMQEGAYRFIRNPNVSAEAIRKAGAMQTVKLAQEFPELLAIEDTTSLSYRHQVAEELGKLGSIQDXSRGWWVHSVLLLEATTFRTVGLLHQEWWMRPDDPADADEKESGKWLAAAATSRLRMGSMMSNVIAVCDREADIHAYLQDKLAHNERFVVRSKHPRKDVESGLYLYDHLKNQPELGGYQISIPQKGVVDKRGKRKNRPARKASLSLRSGRITLKQGNITLNAVLAEEINPPKGETPLKWLLLTSEPVESLAQALRVIDIYTHRWRIEEFHKAWKTGAGAERQRMEEPDNLERMVSILSFVAVRLLQLRESFTLPQALRAQGLLKEAEHVESQSAETVLTPDECQLLGYLDKGKRKRKEKAGSLQWAYMAIARLGGFMDSKRTGIASWGALWEGWEALQSKLDGFLAAKDLMAQGIKI

SEQ ID NO: 7 - protein, 476 aa, unidentified
  REGION 1..476: note = Transposase Tn5
  SITE 119: note = Variant - X = L, M, S, A, V
  SITE 120: note = Variant - X = Y, F, W, E
  SITE 248: note = Variant - X = Y, T, K, S, L, A, W, P, G, R, F, H
MITSALHRAADWAKSVFSSAALGDPRRTARLVNVAAQLAKYSGKSITISSEGSEAMQEGAYRFIRNPNVSAEAIRKAGAMQTVKLAQEFPELLAIEDTTSLSYRHQVAEELGKLGSIQXXSRGWMVHSVLLLEATTFRTVGLLHQEWWMRPDDPADADEKESGKWLAAAATSRLRMGSMMSNVIAVCDREADIHAYLQDKLAHNERFVVRSKHPRKDVESGLYLYDHLKNQPELGGYQISIPQKGVVXKRGKRKNRPARKASLSLRSGRITLKQGNITLNAVLAEEINPPKGETPLKWLLLTSEPVESLAQALRVIDIYTHRWRIEEFHKAWKTGAGAERQRMEEPDNLERMVSILSFVAVRLLQLRESFTLPQALRAQGLLKEAEHVESQSAETVLTPDECQLLGYLDKGKRKRKEKAGSLQWAYMAIARLGGFMDSKRTGIASWGALWEGWEALQSKLDGFLAAKDLMAQGIKI

SEQ ID NO: 8 - protein, 476 aa, unidentified
  REGION 1..476: note = Transposase Tn5
MITSALHRAADWAKSVFSSAALGDPRRTARLVNVAAQLAKYSGKSITISSEGSEAMQEGAYRFIRNPNVSAEAIRKAGAMQTVKLAQEFPELLAIEDTTSLSYRHQVAEELGKLGSIQDKSRGWWVHSVLLLEATTFRTVGLLHQEWWMRPDDPADADEKESGKWLAAAATSRLRMGSMMSNVIAVCDREADIHAYLQDKLAHNERFVVRSRHRRKDVESGLYLYDHLKNQPELGGYQISIPQKGVVDKRGKRKNRPARKASLSLRSGRITLKQGNITLNAVLAEEINPPKGETPLKWLLLTSEPVESLAQALRVIDIYTHRWRIEEFHKAWKTGAGVERQRMEEPDNLERMVSILSFVAVRLLQLRESFTLPQALRAQGLLKEAEHVESQSAETVLTPDECQLLGYLDKGKRKRKEKAGSLQWAYMAIARLGGFMDSKRTGIASWGALWEGWEALQSKLDGFLAAKDLMAQGIKI

SEQ ID NO: 9 - protein, 476 aa, unidentified
  REGION 1..476: note = Transposase Tn5
MITSALHRAADWAKSVFSSAALGDPRRTARLVNVAAQLAKYSGKSITISSEGSEAMQEGAYRFIRNPNVSAEAIRKAGAMQTVKLAQEFPELLAIEDTTSLSYRHQVAEELGKLGSIQDKSRGWWVHSVLLLEATTFRTVGLLHQEWWMRPDDPADADEKESGKWLAAAATSRLRMGSMMSNVIAVCDREADIHAYLQDKLAHNERFVVRSRHRRKDVESGLYLYDHLKNQPELGGYQISIPQKGVVDKRRKRKNRPARKASLSLRSGRITLKQGNITLNAVLAEEINPPKGETPLKWLLLTSEPVESLAQALRVIDIYTHRWRIEEFHKAWKTGAGVERQRMEEPDNLERMVSILSFVAVRLLQLRESFTLPQALRAQGLLKEAEHVESQSAETVLTPDECQLLGYLDKGKRKRKEKAGSLQWAYMAIARLGGFMDSKRTGIASWGALWEGWEALQSKLDGFLAAKDLMAQGIKI

SEQ ID NO: 10 - protein, 476 aa, unidentified
  REGION 1..476: note = Transposase Tn5
MITSALHRAADWAKSVFSSAALGDPRRTARLVNVAAQLAKYSGKSITISSEGSEAMQEGAYRFIRNPNVSAEAIRKAGAMQTVKLAQEFPELLAIEDTTSLSYRHQVAEELGKLGSIQDKSRGWWVHSVLLLEATTFRTVGLLHQQWWMRPDDPADADEKESGKWLAAAATSRLRMGSMMSNVIAVCDRGADIHAYLQDKLAHNERFVVRSKHPRKDVESGLYLYDHLKNQPELGGYQISIPQKGVVDKRRKRKNRPARKASLSLRSGRITLKQGNITLNAVLAEEINPPKGETPLKWLLLTSEPVESLAQALRVIDIYTHRWRIEEFHKAWKTGAGAERQRMEEPDNLERMVSILSFVAVRLLQLRESFTLPQALRAQGLLKEAEHVESQSAETVLTPDECQLLGYLDKGKRKRKEKAGSLQWAYMAIARLGGFMDSKRTGIASWGALWEGWEALQSKLDGFLAAKDLMAQGIKI

SEQ ID NO: 11 - protein, 476 aa, unidentified
  REGION 1..476: note = Transposase Tn5
MITSALHRAADWAKSVFSSAALGDPRRTARLVNVAAQLAKYSGKSITISSEGSKAAQEGAYRFIRNPNVSAEAIRKAGAMQTVKLAQEFPELLAIEDTTSLSYRHQVAEELGKLGSIQDKSRGWWVHSVLLLEATTFRTVGLLHQEWWMRPDDPADADEKESGKWLAAAATSRLRMGSMMSNVIAVCDREADIHAYLQDKLAHNERFVVRSKHPRKDVESGLYLYDHLKNQPELGGYQISIPQKGVVDKRGKRKNRPARKASLSLRSGRITLKQGNITLNAVLAEEINPPKGETPLKWLLLTSEPVESLAQALRVIDIYTHRWRIEEFHKAWKTGAGAERQRMEEPDNLERMVSILSFVAVRLLQLRESFTPPQALRAQGLLKEAEHVESQSAETVLTPDECQLLGYLDKGKRKRKEKAGSLQWAYMAIARLGGFMDSKRTGIASWGALWEGWEALQSKLDGFLAAKDLMAQGIKI

SEQ ID NO: 12 - protein, 476 aa, unidentified
  REGION 1..476: note = Transposase Tn5
  VARIANT 248: note = X = Y, T, K, S, L, A, W, P, G, R, F, H
MITSALHRAADWAKSVFSSAALGDPRRTARLVNVAAQLAKYSGKSITISSEGSKAAQEGAYRFIRNPNVSAEAIRKAGAMQTVKLAQEFPELLAIEDTTSLSYRHQVAEELGKLGSIQDKSRGWWVHSVLLLEATTFRTVGLLHQEWWMRPDDPADADEKESGKWLAAAATSRLRMGSMMSNVIAVCDREADIHAYLQDKLAHNERFVVRSKHPRKDVESGLYLYDHLKNQPELGGYQISIPQKGVVXKRGKRKNRPARKASLSLRSGRITLKQGNITLNAVLAEEINPPKGETPLKWLLLTSEPVESLAQALRVIDIYTHRWRIEEFHKAWKTGAGAERQRMEEPDNLERMVSILSFVAVRLLQLRESFTPPQALRAQGLLKEAEHVESQSAETVLTPDECQLLGYLDKGKRKRKEKAGSLQWAYMAIARLGGFMDSKRTGIASWGALWEGWEALQSKLDGFLAAKDLMAQGIKI

SEQ ID NO: 13 - protein, 476 aa, unidentified
  REGION 1..476: note = Transposase Tn5
  SITE 119: note = Variant - X = L, M, S, A, V
MITSALHRAADWAKSVFSSAALGDPRRTARLVNVAAQLAKYSGKSITISSEGSKAAQEGAYRFIRNPNVSAEAIRKAGAMQTVKLAQEFPELLAIEDTTSLSYRHQVAEELGKLGSIQXKSRGWWVHSVLLLEATTFRTVGLLHQEWWMRPDDPADADEKESGKWLAAAATSRLRMGSMMSNVIAVCDREADIHAYLQDKLAHNERFVVRSKHPRKDVESGLYLYDHLKNQPELGGYQISIPQKGVVDKRGKRKNRPARKASLSLRSGRITLKQGNITLNAVLAEEINPPKGETPLKWLLLTSEPVESLAQALRVIDIYTHRWRIEEFHKAWKTGAGAERQRMEEPDNLERMVSILSFVAVRLLQLRESFTPPQALRAQGLLKEAEHVESQSAETVLTPDECQLLGYLDKGKRKRKEKAGSLQWAYMAIARLGGFMDSKRTGIASWGALWEGWEALQSKLDGFLAAKDLMAQGIKI

SEQ ID NO: 14 - protein, 476 aa, unidentified
  REGION 1..476: note = Transposase Tn5
MITSALHRAADWAKSVFSSAALGDPRRTARLVNVAAQLAKYSGKSITISSEGSKAAQEGAYRFIRNPNVSAEAIRKAGAMQTVKLAQEFPELLAIEDTTSLSYRHQVAEELGKLGSIQDKSRGWMVHSVLLLEATTFRTVGLLHQEWWMRPDDPADADEKESGKWLAAAATSRLRMGSMMSNVIAVCDREADIHAYLQDKLAHNERFVVRSKHPRKDVESGLYLYDHLKNQPELGGYQISIPQKGVVDKRGKRKNRPARKASLSLRSGRITLKQGNITLNAVLAEEINPPKGETPLKWLLLTSEPVESLAQALRVIDIYTHRWRIEEFHKAWKTGAGAERQRMEEPDNLERMVSILSFVAVRLLQLRESFTPPQALRAQGLLKEAEHVESQSAETVLTPDECQLLGYLDKGKRKRKEKAGSLQWAYMAIARLGGFMDSKRTGIASWGALWEGWEALQSKLDGFLAAKDLMAQGIKI

SEQ ID NO: 15 - protein, 477 aa, unidentified
  REGION 1..477: note = Transposase Tn5
MITSALHRAADWAKSVFSSAALGDPRRTARLVNVAAQLAKYSGKSITISSEGSKAAQEGAYRFIRNPNVSAEAIRKAGAMQTVKLAQEFPELLAIEDTTSLSYRHQVAEELGKLGSIQDKSRGWWVHSVLLLEATTFRTVGLLHQEWWMRPDDPADADEKESGKWLAAAATSRLRMGSMMSNVIAVCDREADIHAYLQDKLAHNERFVVRSKHPRKDVESGLYLYDHLKNQPELGGYQISIPQKGVVDVKRGKRKNRPARKASLSLRSGRITLKQGNITLNAVLAEEINPPKGETPLKWLLLTSEPVESLAQALRVIDIYTHRWRIEEFHKAWKTGAGAERQRMEEPDNLERMVSILSFVAVRLLQLRESFTPPQALRAQGLLKEAEHVESQSAETVLTPDECQLLGYLDKGKRKRKEKAGSLQWAYMAIARLGGFMDSKRTGIASWGALWEGWEALQSKLDGFLAAKDLMAQGIKI

SEQ ID NO: 16 - protein, 476 aa, unidentified
  REGION 1..476: note = Transposase Tn5
  SITE 120: note = Variant - X = Y, F, W, E
MITSALHRAADWAKSVFSSAALGDPRRTARLVNVAAQLAKYSGKSITISSEGSKAAQEGAYRFIRNPNVSAEAIRKAGAMQTVKLAQEFPELLAIEDTTSLSYRHQVAEELGKLGSIQDXSRGWWVHSVLLLEATTFRTVGLLHQEWWMRPDDPADADEKESGKWLAAAATSRLRMGSMMSNVIAVCDREADIHAYLQDKLAHNERFVVRSKHPRKDVESGLYLYDHLKNQPELGGYQISIPQKGVVDKRGKRKNRPARKASLSLRSGRITLKQGNITLNAVLAEEINPPKGETPLKWLLLTSEPVESLAQALRVIDIYTHRWRIEEFHKAWKTGAGAERQRMEEPDNLERMVSILSFVAVRLLQLRESFTPPQALRAQGLLKEAEHVESQSAETVLTPDECQLLGYLDKGKRKRKEKAGSLQWAYMAIARLGGFMDSKRTGIASWGALWEGWEALQSKLDGFLAAKDLMAQGIKI

SEQ ID NO: 17 - protein, 476 aa, unidentified
  REGION 1..476: note = Transposase Tn5
  SITE 119: note = Variant - X = L, M, S, A, V
  SITE 120: note = Variant - X = Y, F, W, E
  SITE 248: note = Variant - X = Y, T, K, S, L, A, W, P, G, R, F, H
MITSALHRAADWAKSVFSSAALGDPRRTARLVNVAAQLAKYSGKSITISSEGSKAAQEGAYRFIRNPNVSAEAIRKAGAMQTVKLAQEFPELLAIEDTTSLSYRHQVAEELGKLGSIQXXSRGWMVHSVLLLEATTFRTVGLLHQEWWMRPDDPADADEKESGKWLAAAATSRLRMGSMMSNVIAVCDREADIHAYLQDKLAHNERFVVRSKHPRKDVESGLYLYDHLKNQPELGGYQISIPQKGVVXKRGKRKNRPARKASLSLRSGRITLKQGNITLNAVLAEEINPPKGETPLKWLLLTSEPVESLAQALRVIDIYTHRWRIEEFHKAWKTGAGAERQRMEEPDNLERMVSILSFVAVRLLQLRESFTPPQALRAQGLLKEAEHVESQSAETVLTPDECQLLGYLDKGKRKRKEKAGSLQWAYMAIARLGGFMDSKRTGIASWGALWEGWEALQSKLDGFLAAKDLMAQGIKI

SEQ ID NO: 18 - protein, 476 aa, unidentified
  REGION 1..476: note = Transposase Tn5
MITSALHRAADWAKSVFSSAALGDPRRTARLVNVAAQLAKYSGKSITISSEGSKAAQEGAYRFIRNPNVSAEAIRKAGAMQTVKLAQEFPELLAIEDTTSLSYRHQVAEELGKLGSIQDKSRGWWVHSVLLLEATTFRTVGLLHQEWWMRPDDPADADEKESGKWLAAAATSRLRMGSMMSNVIAVCDREADIHAYLQDKLAHNERFVVRSRHRRKDVESGLYLYDHLKNQPELGGYQISIPQKGVVDKRGKRKNRPARKASLSLRSGRITLKQGNITLNAVLAEEINPPKGETPLKWLLLTSEPVESLAQALRVIDIYTHRWRIEEFHKAWKTGAGVERQRMEEPDNLERMVSILSFVAVRLLQLRESFTPPQALRAQGLLKEAEHVESQSAETVLTPDECQLLGYLDKGKRKRKEKAGSLQWAYMAIARLGGFMDSKRTGIASWGALWEGWEALQSKLDGFLAAKDLMAQGIKI

SEQ ID NO: 19 - protein, 476 aa, unidentified
  REGION 1..476: note = Transposase Tn5
MITSALHRAADWAKSVFSSAALGDPRRTARLVNVAAQLAKYSGKSITISSEGSKAAQEGAYRFIRNPNVSAEAIRKAGAMQTVKLAQEFPELLAIEDTTSLSYRHQVAEELGKLGSIQDKSRGWWVHSVLLLEATTFRTVGLLHQEWWMRPDDPADADEKESGKWLAAAATSRLRMGSMMSNVIAVCDREADIHAYLQDKLAHNERFVVRSRHRRKDVESGLYLYDHLKNQPELGGYQISIPQKGVVDKRRKRKNRPARKASLSLRSGRITLKQGNITLNAVLAEEINPPKGETPLKWLLLTSEPVESLAQALRVIDIYTHRWRIEEFHKAWKTGAGVERQRMEEPDNLERMVSILSFVAVRLLQLRESFTPPQALRAQGLLKEAEHVESQSAETVLTPDECQLLGYLDKGKRKRKEKAGSLQWAYMAIARLGGFMDSKRTGIASWGALWEGWEALQSKLDGFLAAKDLMAQGIKI

SEQ ID NO: 20 - protein, 476 aa, unidentified
  REGION 1..476: note = Transposase Tn5
MITSALHRAADWAKSVFSSAALGDPRRTARLVNVAAQLAKYSGKSITISSEGSKAAQEGAYRFIRNPNVSAEAIRKAGAMQTVKLAQEFPELLAIEDTTSLSYRHQVAEELGKLGSIQDKSRGWWVHSVLLLEATTFRTVGLLHQQWWMRPDDPADADEKESGKWLAAAATSRLRMGSMMSNVIAVCDRGADIHAYLQDKLAHNERFVVRSKHPRKDVESGLYLYDHLKNQPELGGYQISIPQKGVVDKRRKRKNRPARKASLSLRSGRITLKQGNITLNAVLAEEINPPKGETPLKWLLLTSEPVESLAQALRVIDIYTHRWRIEEFHKAWKTGAGAERQRMEEPDNLERMVSILSFVAVRLLQLRESFTPPQALRAQGLLKEAEHVESQSAETVLTPDECQLLGYLDKGKRKRKEKAGSLQWAYMAIARLGGFMDSKRTGIASWGALWEGWEALQSKLDGFLAAKDLMAQGIKI

SEQ ID NO: 21 - skipped

SEQ ID NO: 22 - DNA, 852 bp, Escherichia coli
  source 1..852: mol_type = unassigned DNA
atggctgaaattaccgcatccctggtaaaagagctgcgtgagcgtactggcgcaggcatgatggattgcaaaaaagcactgactgaagctaacggcgacatcgagctggcaatcgaaaacatgcgtaagtccggtgctattaaagcagcgaaaaaagcaggcaacgttgctgctgacggcgtgatcaaaaccaaaatcgacggcaactacggcatcattctggaagttaactgccagactgacttcgttgcaaaagacgctggtttccaggcgttcgcagacaaagttctggacgcagctgttgctggcaaaatcactgacgttgaagttctgaaagcacagttcgaagaagaacgtgttgcgctggtagcgaaaattggtgaaaacatcaacattcgccgcgttgctgcgctggaaggcgacgttctgggttcttatcagcacggtgcgcgtatcggcgttctggttgctgctaaaggcgctgacgaagagctggttaaacacatcgctatgcacgttgctgcaagcaagccagaattcatcaaaccggaagacgtatccgctgaagtggtagaaaaagaataccaggtacagctggatatcgcgatgcagtctggtaagccgaaagaaatcgcagagaaaatggttgaaggccgcatgaagaaattcaccggcgaagtttctctgaccggtcagccgttcgttatggaaccaagcaaaactgttggtcagctgctgaaagagcataacgctgaagtgactggcttcatccgcttcgaagtgggtgaaggcatcgagaaagttgagactgactttgcagcagaagttgctgcgatgtccaagcagtcttaa

SEQ ID NO: 23 - protein, 283 aa, Escherichia coli
MAEITASLVKELRERTGAGMMDCKKALTEANGDIELAIENMRKSGAIKAAKKAGNVAADGVIKTKIDGNYGIILEVNCQTDFVAKDAGFQAFADKVLDAAVAGKITDVEVLKAQFEEERVALVAKIGENINIRRVAALEGDVLGSYQHGARIGVLVAAKGADEELVKHIAMHVAASKPEFIKPEDVSAEVVEKEYQVQLDIAMQSGKPKEIAEKMVEGRMKKFTGEVSLTGQPFVMEPSKTVGQLLKEHNAEVTGFIRFEVGEGIEKVETDFAAEVAAMSKQS

SEQ ID NO: 24 - DNA, 2283 bp, unidentified
  misc_feature 1..2283: note = TS-Tn5 nucleic acid sequence
  source 1..2283: mol_type = unassigned DNA
atggctgaaattaccgcatccctggtaaaagagctgcgtgagcgtactggcgcaggcatgatggattgcaaaaaagcactgactgaagctaacggcgacatcgagctggcaatcgaaaacatgcgtaagtccggtgctattaaagcagcgaaaaaagcaggcaacgttgctgctgacggcgtgatcaaaaccaaaatcgacggcaactacggcatcattctggaagttaactgccagactgacttcgttgcaaaagacgctggtttccaggcgttcgcagacaaagttctggacgcagctgttgctggcaaaatcactgacgttgaagttctgaaagcacagttcgaagaagaacgtgttgcgctggtagcgaaaattggtgaaaacatcaacattcgccgcgttgctgcgctggaaggcgacgttctgggttcttatcagcacggtgcgcgtatcggcgttctggttgctgctaaaggcgctgacgaagagctggttaaacacatcgctatgcacgttgctgcaagcaagccagaattcatcaaaccggaagacgtatccgctgaagtggtagaaaaagaataccaggtacagctggatatcgcgatgcagtctggtaagccgaaagaaatcgcagagaaaatggttgaaggccgcatgaagaaattcaccggcgaagtttctctgaccggtcagccgttcgttatggaaccaagcaaaactgttggtcagctgctgaaagagcataacgctgaagtgactggcttcatccgcttcgaagtgggtgaaggcatcgagaaagttgagactgactttgcagcagaagttgctgcgatgtccaagcagtctggtaccataacttctgctcttcatcgtgcggccgactgggctaaatctgtgttctcttcggcggcgctgggtgatcctcgccgtactgcccgcttggttaacgtcgccgcccaattggcaaaatattctggtaaatcaataaccatctcatcagagggtagtaaagccgcccaggaaggcgcttaccgatttatccgcaatcccaacgtttctgccgaggcgatcagaaaggctggcgccatgcaaacagtcaagttggctcaggagtttcccgaactgctggccattgaggacaccacctctttgagttatcgccaccaggtcgccgaagagcttggcaagctgggctctattcaggataaatcccgcggatggtgggttcactccgttctcttgctcgaggccaccacattccgcaccgtaggattactgcatcaggagtggtggatgcgcccggatgaccctgccgatgcggatgaaaaggagagtggcaaatggctggcagcggccgcaactagccggttacgcatgggcagcatgatgagcaacgtgattgcggtctgtgaccgcgaagccgatattcatgcttatctgcaggacaaactggcgcataacgagcgcttcgtggtgcgctccaagcacccacgcaaggacgtagagtctgggttgtatctgtacgaccatctgaagaaccaaccggagttgggtggctatcagatcagcattccgcaaaagggcgtggtggataaacgcggtaaacgtaaaaatcgaccagcccgcaaggcgagcttgagcctgcgcagtgggcgcatcacgctaaaacaggggaatatcacgctcaacgcggtgctggccgaggagattaacccgcccaagggtgagaccccgttgaaatggttgttgctgaccagcgaaccggtcgagtcgctagcccaagccttgcgcgtcatcgacatttatacccatcgctggcggatcgaggagttccataaggcatggaaaaccggagcaggagccgagaggcaacgcatggaggagccggataatctggagcggatggtctcgatcctctcgtttgttgcggtcaggctgttacagctcagagaaagcttcacgccgccgcaagcactcagggcgcaagggctgctaaaggaagcggaacacgtagaaagccagtccgcagaaacggtgctgaccccggatgaatgtcagctactgggctatctggacaagggaaaacgcaagcgcaaagagaaagcaggtagcttgcagtgggcttacatggcgatagctagactgggcggttttatggacagcaagcgaaccggaattgccagctggggcgccctctgggaaggttgggaagccctgcaaagtaaactggatggctttcttgccgccaaggatctgatggcgcaggggatcaagatctga

SEQ ID NO: 25 - protein, 760 aa, unidentified
  REGION 1..760: note = TS-Tn5 Fusion Protein Amino Acid Sequence
MAEITASLVKELRERTGAGMMDCKKALTEANGDIELAIENMRKSGAIKAAKKAGNVAADGVIKTKIDGNYGIILEVNCQTDFVAKDAGFQAFADKVLDAAVAGKITDVEVLKAQFEEERVALVAKIGENINIRRVAALEGDVLGSYQHGARIGVLVAAKGADEELVKHIAMHVAASKPEFIKPEDVSAEVVEKEYQVQLDIAMQSGKPKEIAEKMVEGRMKKFTGEVSLTGQPFVMEPSKTVGQLLKEHNAEVTGFIRFEVGEGIEKVETDFAAEVAAMSKQSGTITSALHRAADWAKSVFSSAALGDPRRTARLVNVAAQLAKYSGKSITISSEGSKAAQEGAYRFIRNPNVSAEAIRKAGAMQTVKLAQEFPELLAIEDTTSLSYRHQVAEELGKLGSIQDKSRGWWVHSVLLLEATTFRTVGLLHQEWWMRPDDPADADEKESGKWLAAAATSRLRMGSMMSNVIAVCDREADIHAYLQDKLAHNERFVVRSKHPRKDVESGLYLYDHLKNQPELGGYQISIPQKGVVDKRGKRKNRPARKASLSLRSGRITLKQGNITLNAVLAEEINPPKGETPLKWLLLTSEPVESLAQALRVIDIYTHRWRIEEFHKAWKTGAGAERQRMEEPDNLERMVSILSFVAVRLLQLRESFTPPQALRAQGLLKEAEHVESQSAETVLTPDECQLLGYLDKGKRKRKEKAGSLQWAYMAIARLGGFMDSKRTGIASWGALWEGWEALQSKLDGFLAAKDLMAQGIKI

SEQ ID NO: 26 - protein, 760 aa, unidentified
  REGION 1..760: note = TS-Tn mutant protein
MAEITASLVKELRERTGAGMMDCKKALTEANGDIELAIENMRKSGAIKAAKKAGNVAADGVIKTKIDGNYGIILEVNCQTDFVAKDAGFQAFADKVLDAAVAGKITDVEVLKAQFEEERVALVAKIGENINIRRVAALEGDVLGSYQHGARIGVLVAAKGADEELVKHIAMHVAASKPEFIKPEDVSAEVVEKEYQVQLDIAMQSGKPKEIAEKMVEGRMKKFTGEVSLTGQPFVMEPSKTVGQLLKEHNAEVTGFIRFEVGEGIEKVETDFAAEVAAMSKQSGTITSALHRAADWAKSVFSSAALGDPRRTARLVNVAAQLAKYSGKSITISSEGSKAAQEGAYRFIRNPNVSAEAIRKAGAMQTVKLAQEFPELLAIEDTTSLSYRHQVAEELGKLGSIQDKSRGWWVHSVLLLEATTFRTVGLLHQEWWMRPDDPADADEKESGKWLAAAATSRLRMGSMMSNVIAVCDREADIHAYLQDKLAHNERFVVRSRHRRKDVESGLYLYDHLKNQPELGGYQISIPQKGVVDKRRKRKNRPARKASLSLRSGRITLKQGNITLNAVLAEEINPPKGETPLKWLLLTSEPVESLAQALRVIDIYTHRWRIEEFHKAWKTGAGVERQRMEEPDNLERMVSILSFVAVRLLQLRESFTPPQALRAQGLLKEAEHVESQSAETVLTPDECQLLGYLDKGKRKRKEKAGSLQWAYMAIARLGGFMDSKRTGIASWGALWEGWEALQSKLDGFLAAKDLMAQGIKI